European Patent Application EP 4 219 728 A2, published August 2, 2023. Title: ENHANCED DELIVERY OF VIRAL PARTICLES TO THE STRIATUM AND CORTEX. Applicant: Genzyme Corporation. Application EP. The sequence listing filed with the application follows.

SEQUENCE LISTING (1 sequence)

SEQ ID NO: 1 - DNA, 78 bp, synthetic construct
  source 1..78: mol_type = other DNA
cactccctctctgcgcgctcgctcgctcactgaggccgggcgaccaaaggtcgcccacgcccgggctttgcccgggcg